European Patent Application EP 4 438 725 A1, published October 2, 2024. Title: NOVEL PROTEASES AND USES THEREOF. Applicant: CARBIOS. The sequence listing filed with the application follows.

SEQUENCE LISTING (4 sequences)

SEQ ID NO: 1 - protein, 276 aa, synthetic construct [sequence omitted]

SEQ ID NO: 2 - protein, 81 aa, synthetic construct
APAVPVAMAAAGQGVAGQYIVTLKKGVSVDSTVAKRGIRTQHRFGKVLNGFSAKLTDDQLSKLRTTPGVASIEQDAVITVD

SEQ ID NO: 3 - protein, 22 aa, synthetic construct
MKYLLPTAAAGLLLLAAQPAMA

SEQ ID NO: 4 - protein, 8 aa, synthetic construct
LEHHHHHH